European Patent Application EP 4 582 453 A1, published July 9, 2025. Title: 항 CTLA-4 모노클로날 항체 및 이의 용도. Applicant: 주식회사 시클리드. Application KR. The sequence listing filed with the application follows.

SEQUENCE LISTING (48 sequences)

SEQ ID NO: 1 - protein, 5 aa, synthetic construct
NYAMS

SEQ ID NO: 2 - protein, 9 aa, synthetic construct
VIYYDGSNK

SEQ ID NO: 3 - protein, 9 aa, synthetic construct
ARNTYRFDY

SEQ ID NO: 4 - protein, 13 aa, synthetic construct
SGSSSNIGNNAVT

SEQ ID NO: 5 - protein, 7 aa, synthetic construct
SDSNRPS

SEQ ID NO: 6 - protein, 9 aa, synthetic construct
GSWDSSLSG

SEQ ID NO: 7 - protein, 446 aa, synthetic construct
EVQLLESGGGLVQPGGSLRLSCAASGFTFSNYAMSWVRQAPGKGLEWVSVIYYDGSNKYYADSVKGRFTISRDNSKNTLYLQMNSLRAEDTAVYYCARNTYRFDYWGQGTLVTVSSASTKGPSVFPLAPSSKSTSGGTAALGCLVKDYFPEPVTVSWNSGALTSGVHTFPAVLQSSGLYSLSSVVTVPSSSLGTQTYICNVNHKPSNTKVDKKVEPKSCDKTHTCPPCPAPELLGGPSVFLFPPKPKDTLMISRTPEVTCVVVDVSHEDPEVKFNWYVDGVEVHNAKTKPREEQYNSTYRVVSVLTVLHQDWLNGKEYKCKVSNKALPAPIEKTISKAKGQPREPQVYTLPPSRDELTKNQVSLTCLVKGFYPSDIAVEWESNGQPENNYKTTPPVLDSDGSFFLYSKLTVDKSRWQQGNVFSCSVMHEALHNHYTQKSLSLSPGK

SEQ ID NO: 8 - protein, 217 aa, synthetic construct
QSVLTQPPSASGTPGQRVTISCSGSSSNIGNNAVTWYQQLPGTAPKLLIYSDSNRPSGVPDRFSGSKSGTSASLAISGLRSEDEADYYCGSWDSSLSGYVFGGGTKLTVLRTVAAPSVFIFPPSDEQLKSGTASVVCLLNNFYPREAKVQWKVDNALQSGNSQESVTEQDSKDSTYSLSSTLTLSKADYEKHKVYACEVTHQGLSSPVTKSFNRGEC

SEQ ID NO: 9 - protein, 5 aa, synthetic construct
GYSMS

SEQ ID NO: 10 - protein, 9 aa, synthetic construct
SISPSGGNT

SEQ ID NO: 11 - protein, 9 aa, synthetic construct
AKTSELFDY

SEQ ID NO: 12 - protein, 13 aa, synthetic construct
TGSSSNIGSNDVN

SEQ ID NO: 13 - protein, 7 aa, synthetic construct
NDSHRPS

SEQ ID NO: 14 - protein, 9 aa, synthetic construct
GTWDYSLSA

SEQ ID NO: 15 - protein, 446 aa, synthetic construct
EVQLLESGGGLVQPGGSLRLSCAASGFTFSGYSMSWVRQAPGKGLEWVSSISPSGGNTYYADSVKGRFTISRDNSKNTLYLQMNSLRAEDTAVYYCAKTSELFDYWGQGTLVTVSSASTKGPSVFPLAPSSKSTSGGTAALGCLVKDYFPEPVTVSWNSGALTSGVHTFPAVLQSSGLYSLSSVVTVPSSSLGTQTYICNVNHKPSNTKVDKKVEPKSCDKTHTCPPCPAPELLGGPSVFLFPPKPKDTLMISRTPEVTCVVVDVSHEDPEVKFNWYVDGVEVHNAKTKPREEQYNSTYRVVSVLTVLHQDWLNGKEYKCKVSNKALPAPIEKTISKAKGQPREPQVYTLPPSRDELTKNQVSLTCLVKGFYPSDIAVEWESNGQPENNYKTTPPVLDSDGSFFLYSKLTVDKSRWQQGNVFSCSVMHEALHNHYTQKSLSLSPGK

SEQ ID NO: 16 - protein, 217 aa, synthetic construct
QSVLTQPPSASGTPGQRVTISCTGSSSNIGSNDVNWYQQLPGTAPKLLIYNDSHRPSGVPDRFSGSKSGTSASLAISGLRSEDEADYYCGTWDYSLSAYVFGGGTKLTVLRTVAAPSVFIFPPSDEQLKSGTASVVCLLNNFYPREAKVQWKVDNALQSGNSQESVTEQDSKDSTYSLSSTLTLSKADYEKHKVYACEVTHQGLSSPVTKSFNRGEC

SEQ ID NO: 17 - protein, 5 aa, synthetic construct
SYDMS

SEQ ID NO: 18 - protein, 9 aa, synthetic construct
SIYPDNSTI

SEQ ID NO: 19 - protein, 9 aa, synthetic construct
AKSTGLFDY

SEQ ID NO: 20 - protein, 13 aa, synthetic construct
TGSSSNIGSNYVN

SEQ ID NO: 21 - protein, 7 aa, synthetic construct
ADSQRQR

SEQ ID NO: 22 - protein, 9 aa, synthetic construct
GSWDDSLNA

SEQ ID NO: 23 - protein, 446 aa, synthetic construct
EVQLLESGGGLVQPGGSLRLSCAASGFTFSSYDMSWVRQAPGKGLEWVSSIYPDNSTIYYADSVKGRFTISRDNSKNTLYLQMNSLRAEDTAVYYCAKSTGLFDYWGQGTLVTVSSASTKGPSVFPLAPSSKSTSGGTAALGCLVKDYFPEPVTVSWNSGALTSGVHTFPAVLQSSGLYSLSSVVTVPSSSLGTQTYICNVNHKPSNTKVDKKVEPKSCDKTHTCPPCPAPELLGGPSVFLFPPKPKDTLMISRTPEVTCVVVDVSHEDPEVKFNWYVDGVEVHNAKTKPREEQYNSTYRVVSVLTVLHQDWLNGKEYKCKVSNKALPAPIEKTISKAKGQPREPQVYTLPPSRDELTKNQVSLTCLVKGFYPSDIAVEWESNGQPENNYKTTPPVLDSDGSFFLYSKLTVDKSRWQQGNVFSCSVMHEALHNHYTQKSLSLSPGK

SEQ ID NO: 24 - protein, 216 aa, synthetic construct
QSVLTQPPSASGTPGQRVTISCTGSSSNIGSNYVNWYQQLPGTAPKLLIYADSQRQRGPDRFSGSKSGTSASLAISGLRSEDEADYYCGSWDDSLNAYVFGGGTKLTVLRTVAAPSVFIFPPSDEQLKSGTASVVCLLNNFYPREAKVQWKVDNALQSGNSQESVTEQDSKDSTYSLSSTLTLSKADYEKHKVYACEVTHQGLSSPVTKSFNRGEC

SEQ ID NO: 25 - protein, 5 aa, synthetic construct
GYDMS

SEQ ID NO: 26 - protein, 9 aa, synthetic construct
GISPGTGST

SEQ ID NO: 27 - protein, 14 aa, synthetic construct
ARDPTVRTHLWFDY

SEQ ID NO: 28 - protein, 13 aa, synthetic construct
SGSSSNIGNNYVT

SEQ ID NO: 29 - protein, 7 aa, synthetic construct
ADSHRPS

SEQ ID NO: 30 - protein, 9 aa, synthetic construct
GAWDDSLSG

SEQ ID NO: 31 - protein, 451 aa, synthetic construct
EVQLLESGGGLVQPGGSLRLSCAASGFTFSGYDMSWVRQAPGKGLEWVSGISPGTGSTYYADSVKGRFTISRDNSKNTLYLQMNSLRAEDTAVYYCARDPTVRTHLWFDYWGQGTLVTVSSASTKGPSVFPLAPSSKSTSGGTAALGCLVKDYFPEPVTVSWNSGALTSGVHTFPAVLQSSGLYSLSSVVTVPSSSLGTQTYICNVNHKPSNTKVDKKVEPKSCDKTHTCPPCPAPELLGGPSVFLFPPKPKDTLMISRTPEVTCVVVDVSHEDPEVKFNWYVDGVEVHNAKTKPREEQYNSTYRVVSVLTVLHQDWLNGKEYKCKVSNKALPAPIEKTISKAKGQPREPQVYTLPPSRDELTKNQVSLTCLVKGFYPSDIAVEWESNGQPENNYKTTPPVLDSDGSFFLYSKLTVDKSRWQQGNVFSCSVMHEALHNHYTQKSLSLSPGK

SEQ ID NO: 32 - protein, 217 aa, synthetic construct
QSVLTQPPSASGTPGRRVTISCSGSSSNIGNNYVTWYQQLPGTAPKLLIYADSHRPSGVPDRFSGSKSGTSASLAISGLRSEDEADYYCGAWDDSLSGYVFGGGTKLTVLRTVAAPSVFIFPPSDEQLKSGTASVVCLLNNFYPREAKVQWKVDNALQSGNSQESVTEQDSKDSTYSLSSTLTLSKADYEKHKVYACEVTHQGLSSPVTKSFNRGEC

SEQ ID NO: 33 - DNA, 92 bp, synthetic construct
  source 1..92: mol_type = other DNA
attcgatcgatatggagacagacacactcctgctatgggtactgctgctctgggttccaggttccacgtggcagtctgtgctgactcagcca

SEQ ID NO: 34 - DNA, 33 bp, synthetic construct
  source 1..33: mol_type = other DNA
agccaccgtacgtaggaccgtcagcttggtgcc

SEQ ID NO: 35 - DNA, 92 bp, synthetic construct
  source 1..92: mol_type = other DNA
attcgatcgatatggagacagacacactcctgctatgggtactgctgctctgggttccaggttccacgtgggaggtgcagctgttggagtct

SEQ ID NO: 36 - DNA, 33 bp, synthetic construct
  source 1..33: mol_type = other DNA
cttggtgctagctgagctcacggtgaccagtgt

SEQ ID NO: 37 - DNA, 92 bp, synthetic construct; identical to SEQ ID NO: 33
  source 1..92: mol_type = other DNA

SEQ ID NO: 38 - DNA, 33 bp, synthetic construct; identical to SEQ ID NO: 34
  source 1..33: mol_type = other DNA

SEQ ID NO: 39 - DNA, 92 bp, synthetic construct; identical to SEQ ID NO: 35
  source 1..92: mol_type = other DNA

SEQ ID NO: 40 - DNA, 33 bp, synthetic construct; identical to SEQ ID NO: 36
  source 1..33: mol_type = other DNA

SEQ ID NO: 41 - DNA, 92 bp, synthetic construct; identical to SEQ ID NO: 33
  source 1..92: mol_type = other DNA

SEQ ID NO: 42 - DNA, 33 bp, synthetic construct; identical to SEQ ID NO: 34
  source 1..33: mol_type = other DNA

SEQ ID NO: 43 - DNA, 92 bp, synthetic construct; identical to SEQ ID NO: 35
  source 1..92: mol_type = other DNA

SEQ ID NO: 44 - DNA, 33 bp, synthetic construct; identical to SEQ ID NO: 36
  source 1..33: mol_type = other DNA

SEQ ID NO: 45 - DNA, 92 bp, synthetic construct; identical to SEQ ID NO: 33
  source 1..92: mol_type = other DNA

SEQ ID NO: 46 - DNA, 33 bp, synthetic construct; identical to SEQ ID NO: 34
  source 1..33: mol_type = other DNA

SEQ ID NO: 47 - DNA, 92 bp, synthetic construct; identical to SEQ ID NO: 35
  source 1..92: mol_type = other DNA

SEQ ID NO: 48 - DNA, 33 bp, synthetic construct; identical to SEQ ID NO: 36
  source 1..33: mol_type = other DNA